European Patent Specification EP 3 663 408 B1, published May 1, 2024. Title: Sample processing method and sample processing cartridge. Applicant: Qiagen GmbH. The sequence listing filed with the application follows.

SEQUENCE LISTING (9 sequences)

SEQ ID NO: 1 - DNA, 24 bp, Artificial
  FWD primer
cgatgatgctacccctgaaaaact

SEQ ID NO: 2 - DNA, 25 bp, Artificial
  Rev primer
tattgtcgcttgaactgatttcctc

SEQ ID NO: 3 - DNA, 25 bp, Artificial
  Pro probe
cgttgttaagtcaatggaaaacctg

SEQ ID NO: 4 - DNA, 23 bp, Artificial
  FWD primer
aagctccagccacccaaaactac

SEQ ID NO: 5 - DNA, 23 bp, Artificial
  Rev primer
ctaccaaccactaatgcgtcgtc

SEQ ID NO: 6 - DNA, 22 bp, Artificial
  Pro probe
atcgccttccagacgctcaacg

SEQ ID NO: 7 - DNA, 22 bp, Artificial
  FWD primer
gccgctagaggtgaaattcttg

SEQ ID NO: 8 - DNA, 21 bp, Artificial
  Rev primer
cattcttggcaaatgctttcg

SEQ ID NO: 9 - DNA, 21 bp, Artificial
  Pro probe
accggcgcaagacggaccaga